European Patent Application EP 4 176 900 A1, published May 10, 2023. Title: ANTIBODIES DIRECTED AGAINST INTERLEUKIN 36 RECEPTOR (IL-36R). Applicant: AnaptysBio, Inc. The sequence listing filed with the application follows.

SEQUENCE LISTING (58 sequences)

SEQ ID NO: 1 - protein, 116 aa, Artificial Sequence
  Synthetic Sequence
  MISC_FEATURE (4)..(4): Xaa1 is leucine (Leu) or phenylalanine (Phe)
  MISC_FEATURE (5)..(5): Xaa2 is valine (Val), methionine (Met), or leucine (Leu)
  MISC_FEATURE (44)..(44): Xaa3 is arginine (Arg) or glycine (Gly)
  MISC_FEATURE (56)..(56): Xaa4 is glycine (Gly), serine (Ser), or alanine (Ala)
  MISC_FEATURE (72)..(72): Xaa5 is arginine (Arg) or alanine (Ala)
  MISC_FEATURE (74)..(74): Xaa6 is threonine (Thr) or lysine (Lys)
  MISC_FEATURE (84)..(84): Xaa7 is serine (Ser) or alanine (Ala)
  MISC_FEATURE (95)..(95): Xaa8 is tyrosine (Tyr) or phenylalanine (Phe)
QVQXXQSGAEVKKPGASVKVSCKASGFTFTSYDINWVRQAPGQXLEWMGWIYPGDXSTKYNEKFKGRVTITXDXSASTAYMELXSLRSEDTAVYXCTRSFYTMDYWGQGTTVTVSS

SEQ ID NO: 2 - protein, 116 aa, Artificial Sequence
  Synthetic Sequence
QVQLVQSGAEVKKPGASVKVSCKASGFTFTSYDINWVRQAPGQRLEWMGWIYPGDGSTKYNEKFKGRVTITRDTSASTAYMELSSLRSEDTAVYYCTRSFYTMDYWGQGTTVTVSS

SEQ ID NO: 3 - protein, 116 aa, Artificial Sequence
  Synthetic Sequence
QVQLVQSGAEVKKPGASVKVSCKASGFTFTSYDINWVRQAPGQGLEWMGWIYPGDGSTKYNEKFKGRVTITADKSASTAYMELSSLRSEDTAVYFCTRSFYTMDYWGQGTTVTVSS

SEQ ID NO: 4 - protein, 116 aa, Artificial Sequence
  Synthetic Sequence
QVQLMQSGAEVKKPGASVKVSCKASGFTFTSYDINWVRQAPGQRLEWMGWIYPGDSSTKYNEKFKGRVTITRDKSANTAYMELASLRSEDTAVYFCTRSFYTMDYWGQGTTVTVSS

SEQ ID NO: 5 - protein, 116 aa, Artificial Sequence
  Synthetic Sequence
QVQLMQSGAEVKKPGASVKVSCKASGFTFTSYDINWVRQAPGQRLEWMGWIYPGDASTKYNEKFKGRVTITRDKSANTAYMELASLRSEDTAVYFCTRSFYTMDYWGQGTTVTVSS

SEQ ID NO: 6 - protein, 116 aa, Artificial Sequence
  Synthetic Sequence
QVQLMQSGAEVKKPGASVKVSCKASGFTFTSYDINWVRQAPGQRLEWMGWIYPGDSSTKYNEKFKGRVTITADKSANTAYMELASLRSEDTAVYFCTRSFYTMDYWGQGTTVTVSS

SEQ ID NO: 7 - protein, 116 aa, Artificial Sequence
  Synthetic Sequence
QVQLLQSGAEVKKPGASVKVSCKASGFTFTSYDINWVRQAPGQRLEWMGWIYPGDSSTKYNEKFKGRVTITRDKSANTAYMELSSLRSEDTAVYFCTRSFYTMDYWGQGTTVTVSS

SEQ ID NO: 8 - protein, 116 aa, Artificial Sequence
  Synthetic Sequence
QVQLLQSGAEVKKPGASVKVSCKASGFTFTSYDINWVRQAPGQRLEWMGWIYPGDSSTKYNEKFKGRVTITADKSANTAYMELASLRSEDTAVYFCTRSFYTMDYWGQGTTVTVSS

SEQ ID NO: 9 - protein, 116 aa, Artificial Sequence
  Synthetic Sequence
QVQLLQSGAEVKKPGASVKVSCKASGFTFTSYDINWVRQAPGQRLEWMGWIYPGDASTKYNEKFKGRVTITRDKSANTAYMELASLRSEDTAVYFCTRSFYTMDYWGQGTTVTVSS

SEQ ID NO: 10 - protein, 116 aa, Artificial Sequence
  Synthetic Sequence
QVQLLQSGAEVKKPGASVKVSCKASGFTFTSYDINWVRQAPGQRLEWMGWIYPGDSSTKYNEKFKGRVTITRDKSANTAYMELASLRSEDTAVYFCTRSFYTMDYWGQGTTVTVSS

SEQ ID NO: 11 - protein, 116 aa, Artificial Sequence
  Synthetic Sequence
QVQFLQSGAEVKKPGASVKVSCKASGFTFTSYDINWVRQAPGQRLEWMGWIYPGDSSTKYNEKFKGRVTITADKSANTAYMELSSLRSEDTAVYFCTRSFYTMDYWGQGTTVTVSS

SEQ ID NO: 12 - protein, 116 aa, Artificial Sequence
  Synthetic Sequence
QVQFVQSGAEVKKPGASVKVSCKASGFTFTSYDINWVRQAPGQRLEWMGWIYPGDSSTKYNEKFKGRVTITRDKSANTAYMELSSLRSEDTAVYFCTRSFYTMDYWGQGTTVTVSS

SEQ ID NO: 13 - protein, 116 aa, Artificial Sequence
  Synthetic Sequence
QVQFVQSGAEVKKPGASVKVSCKASGFTFTSYDINWVRQAPGQRLEWMGWIYPGDSSTKYNEKFKGRVTITADKSANTAYMELSSLRSEDTAVYFCTRSFYTMDYWGQGTTVTVSS

SEQ ID NO: 14 - protein, 116 aa, Artificial Sequence
  Synthetic Sequence
QVQLLQSGAEVKKPGASVKVSCKASGFTFTSYDINWVRQAPGQRLEWMGWIYPGDSSTKYNEKFKGRVTITRDKSANTAYMELSSLRSEDTAVYYCTRSFYTMDYWGQGTTVTVSS

SEQ ID NO: 15 - protein, 120 aa, Artificial Sequence
  Synthetic Sequence
  MISC_FEATURE (33)..(33): Xaa1 is tryptophan (Trp) or tyrosine (Tyr)
  MISC_FEATURE (35)..(35): Xaa2 is histidine (His), asparagine (Asn), or tyrosine (Tyr)
  MISC_FEATURE (42)..(42): Xaa3 is glycine (Gly) or arginine (Arg)
  MISC_FEATURE (52)..(52): Xaa4 is aspartic acid (Asp), glutamic acid (Glu), or histidine (His)
  MISC_FEATURE (54)..(54): Xaa5 is serine (Ser), threonine (Thr), or tyrosine (Tyr)
  MISC_FEATURE (55)..(55): Xaa6 is asparagine (Asn) or glycine (Gly)
  MISC_FEATURE (56)..(56): Xaa7 is serine (Ser), alanine (Ala), or aspartic acid (Asp)
QVQLVQSGAEVKKPGASVKVSCKASGYTFTNYXMXWVRQAPXQGLEWMGMFXPXXXVTRLNQKFKDRVTMTRDTSTSTVYMELSSLRSEDTAVYYCARTTSMIIGGFAYWGQGTLVTVSS

SEQ ID NO: 16 - protein, 120 aa, Artificial Sequence
  Synthetic Sequence
QVQLVQSGAEVKKPGASVKVSCKASGYTFTNYWMHWVRQAPGQGLEWMGMFDPSNSVTRLNQKFKDRVTMTRDTSTSTVYMELSSLRSEDTAVYYCARTTSMIIGGFAYWGQGTLVTVSS

SEQ ID NO: 17 - protein, 120 aa, Artificial Sequence
  Synthetic Sequence
QVQLVQSGAEVKKPGASVKVSCKASGYTFTNYWMHWVRQAPGQGLEWMGMFEPSNAVTRLNQKFKDRVTMTRDTSTSTVYMELSSLRSEDTAVYYCARTTSMIIGGFAYWGQGTLVTVSS

SEQ ID NO: 18 - protein, 120 aa, Artificial Sequence
  Synthetic Sequence
QVQLVQSGAEVKKPGASVKVSCKASGYTFTNYWMNWVRQAPRQGLEWMGMFEPSNAVTRLNQKFKDRVTMTRDTSTSTVYMELSSLRSEDTAVYYCARTTSMIIGGFAYWGQGTLVTVSS

SEQ ID NO: 19 - protein, 120 aa, Artificial Sequence
  Synthetic Sequence
QVQLVQSGAEVKKPGASVKVSCKASGYTFTNYWMYWVRQAPRQGLEWMGMFHPSNAVTRLNQKFKDRVTMTRDTSTSTVYMELSSLRSEDTAVYYCARTTSMIIGGFAYWGQGTLVTVSS

SEQ ID NO: 20 - protein, 120 aa, Artificial Sequence
  Synthetic Sequence
QVQLVQSGAEVKKPGASVKVSCKASGYTFTNYWMNWVRQAPRQGLEWMGMFHPSNAVTRLNQKFKDRVTMTRDTSTSTVYMELSSLRSEDTAVYYCARTTSMIIGGFAYWGQGTLVTVSS

SEQ ID NO: 21 - protein, 120 aa, Artificial Sequence
  Synthetic Sequence
QVQLVQSGAEVKKPGASVKVSCKASGYTFTNYYMNWVRQAPRQGLEWMGMFHPTGDVTRLNQKFKDRVTMTRDTSTSTVYMELSSLRSEDTAVYYCARTTSMIIGGFAYWGQGTLVTVSS

SEQ ID NO: 22 - protein, 120 aa, Artificial Sequence
  Synthetic Sequence
QVQLVQSGAEVKKPGASVKVSCKASGYTFTNYWMNWVRQAPRQGLEWMGMFHPTGDVTRLNQKFKDRVTMTRDTSTSTVYMELSSLRSEDTAVYYCARTTSMIIGGFAYWGQGTLVTVSS

SEQ ID NO: 23 - protein, 120 aa, Artificial Sequence
  Synthetic Sequence
QVQLVQSGAEVKKPGASVKVSCKASGYTFTNYYMNWVRQAPRQGLEWMGMFHPYGDVTRLNQKFKDRVTMTRDTSTSTVYMELSSLRSEDTAVYYCARTTSMIIGGFAYWGQGTLVTVSS

SEQ ID NO: 24 - protein, 120 aa, Artificial Sequence
  Synthetic Sequence
QVQLVQSGAEVKKPGASVKVSCKASGYTFTNYWMNWVRQAPRQGLEWMGMFHPYGDVTRLNQKFKDRVTMTRDTSTSTVYMELSSLRSEDTAVYYCARTTSMIIGGFAYWGQGTLVTVSS

SEQ ID NO: 25 - protein, 117 aa, Artificial Sequence
  Synthetic Sequence
  MISC_FEATURE (1)..(1): Xaa1 is glutamine (Gln) or aspartic acid (Asp)
  MISC_FEATURE (4)..(4): Xaa2 is leucine (Leu) or phenylalanine (Phe)
  MISC_FEATURE (25)..(25): Xaa3 is threonine (Thr) or serine (Ser)
  MISC_FEATURE (41)..(41): Xaa4 is proline (Pro) or phenylalanine (Phe)
  MISC_FEATURE (44)..(44): Xaa5 is lysine (Lys) or asparagine (Asn)
  MISC_FEATURE (45)..(45): Xaa6 is glycine (Gly) or lysine (Lys)
  MISC_FEATURE (71)..(71): Xaa7 is serine (Ser) or threonine (Thr)
  MISC_FEATURE (72)..(72): Xaa8 is valine (Val) or arginine (Arg)
  MISC_FEATURE (95)..(95): Xaa9 is tyrosine (Tyr) or phenylalanine (Phe)
XVQXQESGPGLVKPSQTLSLTCTVXGYSITSDFAWNWIRQXPGXXLEWIGYISYSGDTNYNPSLKSRVTIXXDTSKNQFSLKLSSVTAADTAVYXCAIRGPYSFTYWGQGTLVTVSS

SEQ ID NO: 26 - protein, 117 aa, Artificial Sequence
  Synthetic Sequence
QVQLQESGPGLVKPSQTLSLTCTVSGYSITSDFAWNWIRQPPGKGLEWIGYISYSGDTNYNPSLKSRVTISVDTSKNQFSLKLSSVTAADTAVYYCAIRGPYSFTYWGQGTLVTVSS

SEQ ID NO: 27 - protein, 117 aa, Artificial Sequence
  Synthetic Sequence
QVQFQESGPGLVKPSQTLSLTCTVSGYSITSDFAWNWIRQPPGKGLEWIGYISYSGDTNYNPSLKSRVTISRDTSKNQFSLKLSSVTAADTAVYFCAIRGPYSFTYWGQGTLVTVSS

SEQ ID NO: 28 - protein, 117 aa, Artificial Sequence
  Synthetic Sequence
QVQLQESGPGLVKPSQTLSLTCTVSGYSITSDFAWNWIRQFPGNKLEWIGYISYSGDTNYNPSLKSRVTISVDTSKNQFSLKLSSVTAADTAVYYCAIRGPYSFTYWGQGTLVTVSS

SEQ ID NO: 29 - protein, 117 aa, Artificial Sequence
  Synthetic Sequence
QVQFQESGPGLVKPSQTLSLTCTVSGYSITSDFAWNWIRQPPGNKLEWIGYISYSGDTNYNPSLKSRVTISRDTSKNQFSLKLSSVTAADTAVYFCAIRGPYSFTYWGQGTLVTVSS

SEQ ID NO: 30 - protein, 117 aa, Artificial Sequence
  Synthetic Sequence
QVQFQESGPGLVKPSQTLSLTCTVSGYSITSDFAWNWIRQFPGKGLEWIGYISYSGDTNYNPSLKSRVTISRDTSKNQFSLKLSSVTAADTAVYFCAIRGPYSFTYWGQGTLVTVSS

SEQ ID NO: 31 - protein, 117 aa, Artificial Sequence
  Synthetic Sequence
QVQFQESGPGLVKPSQTLSLTCTVSGYSITSDFAWNWIRQFPGNKLEWIGYISYSGDTNYNPSLKSRVTISRDTSKNQFSLKLSSVTAADTAVYFCAIRGPYSFTYWGQGTLVTVSS

SEQ ID NO: 32 - protein, 117 aa, Artificial Sequence
  Synthetic Sequence
DVQFQESGPGLVKPSQTLSLTCTVTGYSITSDFAWNWIRQPPGKGLEWIGYISYSGDTNYNPSLKSRVTITRDTSKNQFSLKLSSVTAADTATYFCAIRGPYSFTYWGQGTLVTVSS

SEQ ID NO: 33 - protein, 116 aa, Artificial Sequence
  Synthetic Sequence
QVQLQQSGPELVKPGALVKISCKASGFTFTSYDINWVRQRPGQGLEWIGWIYPGDGSTKYNEKFKGKATLTADKSSSTAYMQLSSLTSENSAVYFCTRSFYTMDYWGQGTSVTVSS

SEQ ID NO: 34 - protein, 120 aa, Artificial Sequence
  Synthetic Sequence
QVQLQQSGPELVRPGASVRMSCKASDYTFTNYWMHWVKQRPGQGLEWIGMFDPSNSVTRLNQKFKDKATLNVDKSSNTAYIQFSSLTFEDSAVYYCARTTSMIIGGFAYWGQGTLVTVSS

SEQ ID NO: 35 - protein, 117 aa, Artificial Sequence
  Synthetic Sequence
DVQFQESGPGLVKPSQSLSLTCTVTGYSITSDFAWNWIRQFPGNKLEWMGYISYSGDTNYNPSLKSRISITRDTSKNQFFLQLNSVTTEDTATYFCAIRGPYSFTYWGPGTLVTVSS

SEQ ID NO: 36 - protein, 112 aa, Artificial Sequence
  Synthetic Sequence
  MISC_FEATURE (34)..(34): Xaa1 is glycine (Gly) or alanine (Ala)
  MISC_FEATURE (41)..(41): Xaa2 is phenylalanine (Phe) or tyrosine (Tyr)
  MISC_FEATURE (54)..(54): Xaa3 is tyrosine (Tyr) or serine (Ser)
DIVMTQSPLSLPVTPGEPASISCRSSKSLLHSNXNTYLYWXLQKPGQSPQLLIXRMSNLASGVPDRFSGSGSGTDFTLKISRVEAEDVGVYYCMQHLEYPFTFGQGTKLEIK

SEQ ID NO: 37 - protein, 112 aa, Artificial Sequence
  Synthetic Sequence
DIVMTQSPLSLPVTPGEPASISCRSSKSLLHSNGNTYLYWYLQKPGQSPQLLIYRMSNLASGVPDRFSGSGSGTDFTLKISRVEAEDVGVYYCMQHLEYPFTFGQGTKLEIK

SEQ ID NO: 38 - protein, 112 aa, Artificial Sequence
  Synthetic Sequence
DIVMTQSPLSLPVTPGEPASISCRSSKSLLHSNGNTYLYWFLQKPGQSPQLLISRMSNLASGVPDRFSGSGSGTDFTLKISRVEAEDVGVYYCMQHLEYPFTFGQGTKLEIK

SEQ ID NO: 39 - protein, 112 aa, Artificial Sequence
  Synthetic Sequence
DIVMTQSPLSLPVTPGEPASISCRSSKSLLHSNANTYLYWFLQKPGQSPQLLISRMSNLASGVPDRFSGSGSGTDFTLKISRVEAEDVGVYYCMQHLEYPFTFGQGTKLEIK

SEQ ID NO: 40 - protein, 112 aa, Artificial Sequence
  Synthetic Sequence
  MISC_FEATURE (32)..(32): Xaa1 is serine (Ser) or arginine (Arg)
  MISC_FEATURE (34)..(34): Xaa2 is glycine (Gly) or alanine (Ala)
  MISC_FEATURE (43)..(43): Xaa3 is glutamine (Gln) or histidine (His)
DIVMTQTPLSLSVTPGQPASISCRSSKSLLHXNXITYFYWYLXKPGQPPQLLIYQMSNLASGVPDRFSGSGSGTDFTLKISRVEAEDVGVYYCAQNLELPLTFGGGTKVEIK

SEQ ID NO: 41 - protein, 112 aa, Artificial Sequence
  Synthetic Sequence
DIVMTQTPLSLSVTPGQPASISCRSSKSLLHSNGITYFYWYLQKPGQPPQLLIYQMSNLASGVPDRFSGSGSGTDFTLKISRVEAEDVGVYYCAQNLELPLTFGGGTKVEIK

SEQ ID NO: 42 - protein, 112 aa, Artificial Sequence
  Synthetic Sequence
DIVMTQTPLSLSVTPGQPASISCRSSKSLLHSNAITYFYWYLQKPGQPPQLLIYQMSNLASGVPDRFSGSGSGTDFTLKISRVEAEDVGVYYCAQNLELPLTFGGGTKVEIK

SEQ ID NO: 43 - protein, 112 aa, Artificial Sequence
  Synthetic Sequence
DIVMTQTPLSLSVTPGQPASISCRSSKSLLHRNAITYFYWYLQKPGQPPQLLIYQMSNLASGVPDRFSGSGSGTDFTLKISRVEAEDVGVYYCAQNLELPLTFGGGTKVEIK

SEQ ID NO: 44 - protein, 112 aa, Artificial Sequence
  Synthetic Sequence
DIVMTQTPLSLSVTPGQPASISCRSSKSLLHRNAITYFYWYLHKPGQPPQLLIYQMSNLASGVPDRFSGSGSGTDFTLKISRVEAEDVGVYYCAQNLELPLTFGGGTKVEIK

SEQ ID NO: 45 - protein, 107 aa, Artificial Sequence
  Synthetic Sequence
  MISC_FEATURE (64)..(64): Xaa1 is serine (Ser) or proline (Pro)
  MISC_FEATURE (71)..(71): Xaa2 is phenylalanine (Phe) or tyrosine (Tyr)
DIQMTQSPSSLSASVGDRVTITCRASQDINNYLNWYQQKPGKAPKLLIYYTSRLHSGVPSRFSXSGSGTDXTFTISSLQPEDIATYYCQQGHTLPWTFGGGTKVEIK

SEQ ID NO: 46 - protein, 107 aa, Artificial Sequence
  Synthetic Sequence
DIQMTQSPSSLSASVGDRVTITCRASQDINNYLNWYQQKPGKAPKLLIYYTSRLHSGVPSRFSGSGSGTDFTFTISSLQPEDIATYYCQQGHTLPWTFGGGTKVEIK

SEQ ID NO: 47 - protein, 107 aa, Artificial Sequence
  Synthetic Sequence
DIQMTQSPSSLSASVGDRVTITCRASQDINNYLNWYQQKPGKAPKLLIYYTSRLHSGVPSRFSPSGSGTDYTFTISSLQPEDIATYYCQQGHTLPWTFGGGTKVEIK

SEQ ID NO: 48 - protein, 112 aa, Artificial Sequence
  Synthetic Sequence
DIVMTQAAPSVPVTPGESVSISCRSSKSLLHSNGNTYLYWFLQRPGQSPQLLISRMSNLASGVPDRFSGSGSGTAFTLRISRVEAEDVGVYYCMQHLEYPFTFGSGTKLEIK

SEQ ID NO: 49 - protein, 112 aa, Artificial Sequence
  Synthetic Sequence
DIVMTQAAFSNPVTLGTSASISCRSSKSLLHSNGITYFYWYLQRPGQSPQLLIYQMSNLASGVPDRFSGSGSGTDFTLRISRVEAEDVGIYYCAQNLELPLTFGAGTKLELK

SEQ ID NO: 50 - protein, 107 aa, Artificial Sequence
  Synthetic Sequence
DIQMTQTTSSLSASLGDRVTINCRASQDINNYLNWYQQKPDGTIRLLIYYTSRLHSGVPSRFSPNGSGTDYSLTINNLEQEDIATYFCQQGHTLPWTFGGGTKLEIK

SEQ ID NO: 51 - protein, 117 aa, Artificial Sequence
  Synthetic Sequence
DVQFQESGPGLVKPSQTLSLTCTVTGYSITSDFAWNWIRQPPGKGLEWIGYISYSGDTNYNPSLKSRVTITRDTSKNQFSLKLSSVTAADTAVYFCAIRGPYSFTYWGQGTLVTVSS

SEQ ID NO: 52 - protein, 118 aa, Artificial Sequence
  Synthetic Sequence
DVQFQESGPGLVKPSQTLSLTCTVTGYSITADFAWNWIRQPPGKGLEWIGYISYSGDTNYNPSLKSRVTITRDTSKNQFSLKLSSVTAADTAVYFCAIRGPYSFTYWGQGTLVTVSSA

SEQ ID NO: 53 - protein, 118 aa, Artificial Sequence
  Synthetic Sequence
DLQFQESGPGLVKPSQTLSLTCTVTGYSITADFAWNWIRQPPGKGLEWIGYISYSGDTNYNPSLKSRVTITRDTSKNQFSLKLSSVTAADTAVYFCAIRGPYSFTYWGQGTLVTVSSA

SEQ ID NO: 54 - protein, 118 aa, Artificial Sequence
  Synthetic Sequence
DLQFQESGPGLVKPSQTLSLTCTVSRYSITADFAWNWIRQPPGKGLEWIGYISYSGDTNYNPSLKSRVTITRDTSKNQFSLKLSSVTAADTAVYFCAIRGPYSFTYWGQGTLVTVSSA

SEQ ID NO: 55 - protein, 109 aa, Artificial Sequence
  Synthetic Sequence
DIQMTQSPSSLSASVGDRVTITCRASQWINNYLNWYQQKPGKAPKLLIYYTSMLHSGVPSRFSPSGSGNDYTFTISSLQPEDIATYYCQQGHTLPWTFGGGTKVEIKRT

SEQ ID NO: 56 - protein, 116 aa, Artificial Sequence
  Synthetic Sequence
  MISC_FEATURE (4)..(4): Xaa1 is leucine (Leu) or phenylalanine (Phe)
  MISC_FEATURE (5)..(5): Xaa2 is valine (Val), methionine (Met), or leucine (Leu)
  MISC_FEATURE (44)..(44): Xaa3 is arginine (Arg) or glycine (Gly)
  MISC_FEATURE (56)..(56): Xaa4 is glycine (Gly), serine (Ser), or alanine (Ala)
  MISC_FEATURE (72)..(72): Xaa5 is arginine (Arg) or alanine (Ala)
  MISC_FEATURE (74)..(74): Xaa6 is threonine (Thr) or lysine (Lys)
  MISC_FEATURE (77)..(77): Xaa7 is serine (Ser) or asparagine (Asn)
  MISC_FEATURE (84)..(84): Xaa8 is serine (Ser) or alanine (Ala)
  MISC_FEATURE (95)..(95): Xaa9 is tyrosine (Tyr) or phenylalanine (Phe)
QVQXXQSGAEVKKPGASVKVSCKASGFTFTSYDINWVRQAPGQXLEWMGWIYPGDXSTKYNEKFKGRVTITXDXSAXTAYMELXSLRSEDTAVYXCTRSFYTMDYWGQGTTVTVSS

SEQ ID NO: 57 - protein, 118 aa, Artificial Sequence
  Synthetic Sequence
  MISC_FEATURE (1)..(1): Xaa1 is glutamine (Gln) or aspartic acid (Asp)
  MISC_FEATURE (2)..(2): Xaa2 is valine (Val) or leucine (Leu)
  MISC_FEATURE (4)..(4): Xaa3 is leucine (Leu) or phenylalanine (Phe)
  MISC_FEATURE (25)..(25): Xaa4 is threonine (Thr) or serine (Ser)
  MISC_FEATURE (26)..(26): Xaa5 is glycine (Gly) or arginine (Arg)
  MISC_FEATURE (31)..(31): Xaa6 serine (Ser) or alanine (Ala)
  MISC_FEATURE (41)..(41): Xaa7 is proline (Pro) or phenylalanine (Phe)
  MISC_FEATURE (44)..(44): Xaa8 is lysine (Lys) or asparagine (Asn)
  MISC_FEATURE (45)..(45): Xaa9 is glycine (Gly) or lysine (Lys)
  MISC_FEATURE (71)..(71): Xaa10 is serine (Ser) or threonine (Thr)
  MISC_FEATURE (72)..(72): Xaa11 is valine (Val) or arginine (Arg)
  MISC_FEATURE (93)..(93): Xaa12 is threonine (Thr) or valine (Val)
  MISC_FEATURE (95)..(95): Xaa13 is tyrosine (Tyr) or phenylalanine (Phe)
  MISC_FEATURE (118)..(118): Xaa14 is is alanine (Ala) or absent
XXQXQESGPGLVKPSQTLSLTCTVXXYSITXDFAWNWIRQXPGXXLEWIGYISYSGDTNYNPSLKSRVTIXXDTSKNQFSLKLSSVTAADTAXYXCAIRGPYSFTYWGQGTLVTVSSX

SEQ ID NO: 58 - protein, 109 aa, Artificial Sequence
  Synthetic Sequence
  MISC_FEATURE (28)..(28): Xaa1 is aspartic acid (Asp) or tryptophan (Trp)
  MISC_FEATURE (53)..(53): Xaa2 is arginine (Arg) or methionine (Met)
  MISC_FEATURE (64)..(64): Xaa3 is glycine (Gly), serine (Ser) or proline (Pro)
  MISC_FEATURE (69)..(69): Xaa4 is threonine (Thr) or asparagine (Asn)
  MISC_FEATURE (71)..(71): Xaa5 is phenylalanine (Phe) or tyrosine (Tyr)
  MISC_FEATURE (108)..(108): Xaa6 is arginine (Arg) or absent
  MISC_FEATURE (109)..(109): Xaa7 is threonine (Thr) or absent
DIQMTQSPSSLSASVGDRVTITCRASQXINNYLNWYQQKPGKAPKLLIYYTSXLHSGVPSRFSXSGSGXDXTFTISSLQPEDIATYYCQQGHTLPWTFGGGTKVEIKXX